European Patent Application EP 4 129 280 A1, published February 8, 2023. Title: APPLICATION OF THYROID HORMONES AND ITS ANALOGUES IN PREPARATION OF DRUGS FOR TREATING ALPHA-THALASSEMIA. Applicant: Ruijin Hospital Affiliated to Shanghai Jiao Tong University School of Medicine. The sequence listing filed with the application follows.

SEQUENCE LISTING (30 sequences)

SEQ ID NO: 1 - DNA, 429 bp, humanζ- Globin gene sequence(2 Ambystoma laterale x Ambystoma jeffersonianum)
atgtctctgaccaagactgagaggaccatcattgtgtccatgtgggccaagatctccacgcaggccgacaccatcggcaccgagactctggagaggctcttcctcagccacccgcagaccaagacctacttcccgcacttcgacctgcacccggggtccgcgcagttgcgcgcgcacggctccaaggtggtggccgccgtgggcgacgcggtgaagagcatcgacgacatcggcggcgccctgtccaagctgagcgagctgcacgcctacatcctgcgcgtggacccggtcaacttcaagctcctgtcccactgcctgctggtcaccctggccgcgcgcttccccgccgacttcacggccgaggcccacgccgcctgggacaagttcctatcggtcgtatcctctgtcctgaccgagaagtaccgctga

SEQ ID NO: 2 - DNA, 18 bp, Human-β-actin-F(2 Ambystoma laterale x Ambystoma jeffersonianum)
ccaaccgcgagaagatga

SEQ ID NO: 3 - DNA, 20 bp, Human-β-actin-R(2 Ambystoma laterale x Ambystoma jeffersonianum)
ccagaggcgtacagggatag

SEQ ID NO: 4 - DNA, 17 bp, Human-HBA1/2-F(2 Ambystoma laterale x Ambystoma jeffersonianum)
aaggtcggcgcgcacgc

SEQ ID NO: 5 - DNA, 18 bp, Human-HBA1/2-R(2 Ambystoma laterale x Ambystoma jeffersonianum)
ctcaggtcgaagtgcggg

SEQ ID NO: 6 - DNA, 21 bp, Human-HBZ-F(2 Ambystoma laterale x Ambystoma jeffersonianum)
ggaccatcattgtgtccatgt

SEQ ID NO: 7 - DNA, 21 bp, Human-HBZ-R(2 Ambystoma laterale x Ambystoma jeffersonianum)
gggaagtaggtcttggtctgc

SEQ ID NO: 8 - DNA, 20 bp, Human-HBE1-F(2 Ambystoma laterale x Ambystoma jeffersonianum)
tgcatgtggatcctgagaac

SEQ ID NO: 9 - DNA, 19 bp, Human-HBE1-R(2 Ambystoma laterale x Ambystoma jeffersonianum)
cgacagcagacaccagctt

SEQ ID NO: 10 - DNA, 20 bp, Human-HBG1/2-F(2 Ambystoma laterale x Ambystoma jeffersonianum)
agcacctggatgatctcaag

SEQ ID NO: 11 - DNA, 20 bp, Human-HBG1/2-R(2 Ambystoma laterale x Ambystoma jeffersonianum)
aaacggtcaccagcacattt

SEQ ID NO: 12 - DNA, 19 bp, Human-HBD-F(2 Ambystoma laterale x Ambystoma jeffersonianum)
gatgcagttggtggtgagg

SEQ ID NO: 13 - DNA, 19 bp, Human-HBD-R(2 Ambystoma laterale x Ambystoma jeffersonianum)
gggttgcccataacagcat

SEQ ID NO: 14 - DNA, 20 bp, Human-HBB-F(2 Ambystoma laterale x Ambystoma jeffersonianum)
gcacgtggatcctgagaact

SEQ ID NO: 15 - DNA, 20 bp, Human-HBB-R(2 Ambystoma laterale x Ambystoma jeffersonianum)
cactggtggggtgaattctt

SEQ ID NO: 16 - DNA, 432 bp, Zebrafish zebrafish zeta-globin gene sequence(2 Ambystoma laterale x Ambystoma jeffersonianum)
atgagtctttctgctaaagacaaggccgccgtgaggggcttctgggccaagattgccccaaagggagagcaaattggtaacgaggcgttttccagattgcttttggtgtaccctcagaccaagacctacttctcccactggaacgatctggcccccggctctccctctgtgaagaagcagggaaagaagatcgtcggtggactcggtctggctgttgataaaatcgacgaccttttcaacggcctgctgaacctcagtgaattgcacgcctttcagctgagagtcgaccctgctaacttcaagctcctgtctcactgtctgctggtggtgttcgccatgctcttccctgatgacttcaccgctgaggtccatctggccatcgacaagttcctggcaagagtggctttggctctgtctgacaaatatcgttaa

SEQ ID NO: 17 - DNA, 20 bp, Zebrafish-β-actin-F(2 Ambystoma laterale x Ambystoma jeffersonianum)
tgctgttttcccctccattg

SEQ ID NO: 18 - DNA, 19 bp, Zebrafish-β-actin-R(2 Ambystoma laterale x Ambystoma jeffersonianum)
ttctgtcccatgccaacca

SEQ ID NO: 19 - DNA, 21 bp, Zebrafish-hbae1-F(2 Ambystoma laterale x Ambystoma jeffersonianum)
ctgaggctgtcagcaaaatcg

SEQ ID NO: 20 - DNA, 21 bp, Zebrafish-hbae1-R(2 Ambystoma laterale x Ambystoma jeffersonianum)
gaacaaagtggccagaaccac

SEQ ID NO: 21 - DNA, 21 bp, Zebrafish-hbae3-F(2 Ambystoma laterale x Ambystoma jeffersonianum)
gctgatggatgacctgaaggg

SEQ ID NO: 22 - DNA, 21 bp, Zebrafish-hbae3-R(2 Ambystoma laterale x Ambystoma jeffersonianum)
ctcaggagtgaagtcgtctgg

SEQ ID NO: 23 - DNA, 21 bp, Zebrafish-hbae5-F(2 Ambystoma laterale x Ambystoma jeffersonianum)
tgctgaacctcagtgaattgc

SEQ ID NO: 24 - DNA, 21 bp, Zebrafish-hbae5-R(2 Ambystoma laterale x Ambystoma jeffersonianum)
ggaacttgtcgatggccagat

SEQ ID NO: 25 - DNA, 20 bp, Zebrafish-hbbe1-F(2 Ambystoma laterale x Ambystoma jeffersonianum)
tccacgtagatcccgacaac

SEQ ID NO: 26 - DNA, 20 bp, Zebrafish-hbbe1-R(2 Ambystoma laterale x Ambystoma jeffersonianum)
tactgtcttcccagagcgga

SEQ ID NO: 27 - DNA, 21 bp, Zebrafish-hbbe2-F(2 Ambystoma laterale x Ambystoma jeffersonianum)
ggactggacagagccatgaag

SEQ ID NO: 28 - DNA, 21 bp, Zebrafish-hbbe2-R(2 Ambystoma laterale x Ambystoma jeffersonianum)
gaggcaatcacgattgtcagg

SEQ ID NO: 29 - DNA, 20 bp, Zebrafish-hbbe3-F(2 Ambystoma laterale x Ambystoma jeffersonianum)
ttgtgtggacagctgaggag

SEQ ID NO: 30 - DNA, 20 bp, Zebrafish-hbbe3-R(2 Ambystoma laterale x Ambystoma jeffersonianum)
acggatagacgaccaagcat